European Patent Specification EP 3 452 579 B1, published October 23, 2024. Title: Transglutaminase Mediated High Molecular Weight Hyaluronan Hydrogels. Applicant: ETH Zuerich. The sequence listing filed with the application follows.

SEQUENCE LISTING (39 sequences)

SEQ ID NO: 1 - protein, 8 aa, Homo sapiens
  MOD_RES (1)..(1): ACETYLATION
  MOD_RES (1)..(1): ACETYLATION
  MOD_RES (5)..(5): AMIDATION
FKGGERCG

SEQ ID NO: 2 - protein, 5 aa, Homo sapiens
  MOD_RES (1)..(1): ACETYLATION
  MOD_RES (5)..(5): AMIDATION
FKGGC

SEQ ID NO: 3 - protein, 8 aa, Homo sapiens
  MOD_RES (1)..(1): ACETYLATION
FKGGERCG

SEQ ID NO: 4 - protein, 5 aa, Homo sapiens
  MOD_RES (1)..(1): ACETYLATION
FKGGC

SEQ ID NO: 5 - protein, 5 aa, Homo sapiens
  MOD_RES (1)..(1): ACETYLATION
LKGGC

SEQ ID NO: 6 - protein, 4 aa, Homo sapiens
  MISC_FEATURE (1)..(1): Dopa (L-3,4-dihydroxyphenylalanine)
  MOD_RES (1)..(1): ACETYLATION
XKGC

SEQ ID NO: 7 - protein, 16 aa, Homo sapiens
  MOD_RES (1)..(1): ACETYLATION
  MOD_RES (16)..(16): AMIDATION
FKGGGPQGIWGQERCG

SEQ ID NO: 8 - protein, 16 aa, Homo sapiens
  MOD_RES (1)..(1): ACETYLATION
  MOD_RES (16)..(16): AMIDATION
FKGGGPQGIAGQERCG

SEQ ID NO: 9 - protein, 13 aa, Homo sapiens
  MOD_RES (1)..(1): ACETYLATION
FKGGGPQGIWGQC

SEQ ID NO: 10 - protein, 13 aa, Homo sapiens
  MOD_RES (1)..(1): ACETYLATION
FKGGGPQGIAGQC

SEQ ID NO: 11 - protein, 4 aa, Homo sapiens
  MOD_RES (1)..(1): ACETYLATION
  MOD_RES (4)..(4): AMIDATION
FKGC

SEQ ID NO: 12 - protein, 4 aa, Homo sapiens
  MOD_RES (1)..(1): ACETYLATION
FKGC

SEQ ID NO: 13 - protein, 4 aa, Homo sapiens
  MOD_RES (1)..(1): ACETYLATION
  MOD_RES (4)..(4): AMIDATION
LKGC

SEQ ID NO: 14 - protein, 4 aa, Homo sapiens
  MOD_RES (1)..(1): ACETYLATION
LKGC

SEQ ID NO: 15 - protein, 8 aa, Homo sapiens
NQEQVSPL

SEQ ID NO: 16 - protein, 4 aa, Homo sapiens
QQLG

SEQ ID NO: 17 - protein, 11 aa, Homo sapiens
GQLKHLEQQEG

SEQ ID NO: 18 - protein, 9 aa, Homo sapiens
NQEQVSPLC

SEQ ID NO: 19 - protein, 12 aa, Homo sapiens
NQEQVSPLERCG

SEQ ID NO: 20 - protein, 20 aa, Homo sapiens
NQEQVSPLGPQGIWGQERCG

SEQ ID NO: 21 - protein, 15 aa, Homo sapiens
NQEQVSPLGGGERCG

SEQ ID NO: 22 - protein, 12 aa, Homo sapiens
NQEQVSPLDRCG

SEQ ID NO: 23 - protein, 7 aa, Homo sapiens
  MOD_RES (1)..(1): ACETYLATION
  MOD_RES (5)..(5): AMIDATION
GQQQLGC

SEQ ID NO: 24 - protein, 10 aa, Homo sapiens
GQQQLGERCG

SEQ ID NO: 25 - protein, 10 aa, Homo sapiens
GQQQLGDRCG

SEQ ID NO: 26 - protein, 7 aa, Homo sapiens
GQQQLGC

SEQ ID NO: 27 - protein, 12 aa, Homo sapiens
GQLKHLEQQEGC

SEQ ID NO: 28 - protein, 15 aa, Homo sapiens
GQLKHLEQQEGERCG

SEQ ID NO: 29 - protein, 15 aa, Homo sapiens
GQLKHLEQQEGDRCG

SEQ ID NO: 30 - DNA, 19 bp, Homo sapiens
aagtaccaggcagtgacag

SEQ ID NO: 31 - DNA, 20 bp, Homo sapiens
cctgtttccgtagcctcatg

SEQ ID NO: 32 - DNA, 19 bp, Homo sapiens
cagccgcttcacctacagc

SEQ ID NO: 33 - DNA, 23 bp, Homo sapiens
ttttgtattcaatcactgtcgcc

SEQ ID NO: 34 - DNA, 21 bp, Homo sapiens
ggaattcggtgtggacatagg

SEQ ID NO: 35 - DNA, 20 bp, Homo sapiens
acttgggtcctttgggtttg

SEQ ID NO: 36 - DNA, 21 bp, Homo sapiens
attcctagtggctccaatgtg

SEQ ID NO: 37 - DNA, 21 bp, Homo sapiens
gcctacctccatatgcatttt

SEQ ID NO: 38 - DNA, 21 bp, Homo sapiens
gaatgggaaccagcctatacc

SEQ ID NO: 39 - DNA, 22 bp, Homo sapiens
tctgtactttcctctgttgctg